European Patent Application EP 4 772 629 A1, published July 8, 2026. Title: 含有硫代磷酸酯键的RNA及其制备方法. Applicant: 吉林凯莱英医药化学有限公司. The sequence listing filed with the application follows.

SEQUENCE LISTING (31 sequences)

SEQ ID NO: 1 - protein, 374 aa, Escherichia phage T4
MQELFNNLMELCKDSQRKFFYSDDVSASGRTYRIFSYNYASYSDWLLPDALECRGIMFEMDGEKPVRIASRPMEKFFNLNENPFTMNIDLNDVDYILTKEDGSLVSTYLDGDEILFKSKGSIKSEQALMANGILMNINHHRLRDRLKELAEDGFTANFEFVAPTNRIVLAYQEMKIILLNVRENETGEYISYDDIYKDATLRPYLVERYEIDSPKWIEEAKNAENIEGYVAVMKDGSHFKIKSDWYVSLHSTKSSLDNPEKLFKTIIDGASDDLKAMYADDEYSYRKIEAFETTYLKYLDRALFLVLDCHNKHCGKDRKTYAMEAQGVAKGAGMDHLFGIIMSLYQGYDSQEKVMCEIEQNFLKNYKKFIPEGY

SEQ ID NO: 2 - protein, 335 aa, Salmonella phage STP4-a
MFKKYSSLENHYNNKFISKIRFEGKDGGLWVAREKIHGTNFSIIVSKDSVSACKRSGPILPSESFYGHEIILKNYDESIKTIQRCMNANELGSVSSYQIFGEFAGQGIQKEVDYGEKDFYVFDILVNTQNGNVLYMDDMMMTSFCNEFGFKMAPFIGCGSFDELIQLPNNFTSVIKAYNEAAKDDLKEVNLCVFDPLVTDDNVAEGYVLKPVYPDFFNNGTRIAIKSKNSRFTEKKKSDKPIKPKAVLTSNDSTVLANLCEYSTWNRVSNVISHIGEVKAKDFGKVMGLTIQDIFIEAKREGVDIVHADNPDLVKRELQTVVSNTIREKWLEIVS

SEQ ID NO: 3 - protein, 334 aa, Escherichia phage T4
MFKKYSSLENHYNSKFIEKLYSLGLTGGEWVAREKIHGTNFSLIIERDKVTCAKRTGPILPAEDFFGYEIILKNYADSIKAVQDIMETSAVVSYQVFGEFAGPGIQKNVDYCDKDFYVFDIIVTTESGDVTYVDDYMMESFCNTFKFKMAPLLGRGKFEELIKLPNDLDSVVQDYNFTVDHAGLVDANKCVWNAEAKGEVFTAEGYVLKPCYPSWLRNGNRVAIKCKNSKFSEKKKSDKPIKAKVELSEADNKLVGILACYVTLNRVNNVISKIGEIGPKDFGKVMGLTVQDILEETSREGITLTQADNPSLIKKELVKMVQDVLRPAWIELVS

SEQ ID NO: 4 - protein, 335 aa, Vibrio phage KVP40
MSFVKYTSLENSYRQAFVDKCDMLGVREWVALEKIHGANFSFIVEFKPNEAQDGAEFTVTPAKRTSTIGANVMGDYDFYGCTSVVEAHTAKMEAISNWLWARGIINVGETIIVYGELAGKGVQKEVNYGDKDFWAYDILLPETGKFLDWDVVLEACEFAKVKTTHEIARGTLDELLRIDPLFRSFHTPADVDGDNVAEGFVVKQLRNEKRLHNGSRAILKVKNDKFKEKKNKAGKTPRAAVVLTEEQEKLHAAFSCYLTENRLRNVLSKLETVTQKQFGMISGLFIKDAKDEFERDELNETAIARDDWDVIKRSLTNIANEILRKNWLDILDGNF

SEQ ID NO: 5 - protein, 334 aa, Yersinia phage fPS-2
MFKKYSSLENHYNSKFIEKLYSLGLTGGEWVAREKIHGTNFSLIIERDKVTCAKRTGPILPAEDFFGYEIILKNYADSIKAVQDIMETSAVVSYQVFGEFAGPGIQKNVDYGDKDFYVFDIIVTTESGGVTYVDDYMMESFCNSFGFKIAPLLGRGKFEDLIKLPNDLDSVVQDYNFTVDHAGLVDANKCVWNAEAKGEVFTAEGYVLKPCYPSWLPNRNRVAIKCKNSKFSEKKKSDKPIKAKVELSEADNKLVGILACYVTLNRVNNVISKIGEIGPKDFGKVMGLTVQDILEETSREGITLTQADNPSLIKKELVKMVQDVLRPAWIELVS

SEQ ID NO: 6 - protein, 327 aa, Vibrio phage nt-1
MSFVKYTSLENSYRQAFVDKCDMLGVRDWVALEKIHGANFSFIVEFDGGYTVTPAKRTSIIGATATGDYDFYGCTSVVEAHKEKVELVANFLWLNEYINLYEPIIIYGELAGKGIQKEVNYGDKDFWAFDIFLPQREEFVDWDTCVAAFTNAEIKYTKELARGTLDELLRIDPLFKSLHTPAEHEGDNVAEGFVVKQLHSEKRLQSGSRAILKVKNEKFKEKKKKEGKTPTKLVLTPEQEKLHAEFSCYLTENRLKNVLSKLGTVNQKQFGMISGLFVKDAKDEFERDELNEVAIDRDDWNAIRRSLTNIANEILRKNWLNILDGNF

SEQ ID NO: 7 - protein, 374 aa, Shigella phage Sf22
MQELFNNLMELCKDSQRKFFYSDDVSASGRTYRIFSYNYASYSDWLLPDALECRGIMFEMDGEKPVRIASRPMEKFFNLNENPFTMNIDLNDVDYILTKEDGSLVSTYLDGDEILFKSKGSIKSEQALMANGILMNINHHQLRDRLKELAEDGFTANFEFVAPTNRIVLAYQEMKIILLNIRENETGEYISYDDIYKDAALRPYLVERFEVDSPKWIEEAKNAENIEGYVAVMKDGSHFKIKSDWYVSLHSTKSSLDNPEKLFKTIIDGASDDLKAMYADDEYSYRKIEAFETTYLKYLDRALFLVLDCHNKHCGKDRKTYAMEAQGVAKGAGMEHLFGIIMSLYQGYDSQEKVMCEIEQNFLKNYKKFIPEGY

SEQ ID NO: 8 - protein, 381 aa, Vibrio phage VH7D
MNVQELYKNLMSLADDAEGKFFFADHLSPLGEKFRVFSYHIASYSDWLLPGALEARGIMFQLDDNDEMIRIVSRPMEKFFNLNENPFTMELDLTTTVQLMDKADGSLISTYLSGENFALKSKTSIFSEQAVAANRYIKKPENRDLWEFCDDCTQAGLTVNMEWCAPNNRIVLEYPEAKLVILNIRDNETGDYVSFDDIPQSALMRVKQWLVDEYDPATAHEPDFVEKLRDTKGIEGMILRLANGQSVKIKTQWYVDLHSQKDSVNVPKKLVTTILNGNHDDLYALFADDKPTIERIREFDSHVTKTLTNSFNAVRQFYARNRHLARKDYAIAGQKVLKPWEFGVAMIAYQKQTVEGVYESLVTAYLKRPELAIPEKYLNGV

SEQ ID NO: 9 - protein, 335 aa, Bacteriophage dhaeg
MFKKYSSLENHYNSKFIEKLRTNGLTGGEWVAREKIHGTNFSLIIERDAVTCAKRTGPILPAEDFYGYEIVLKNYADSIKSIQDIMETSAAVSYQVFGEFAGTGIQKNVDYGDKDFYVFDIIVTTESGDVTYVDDYMMESFCKTFKFKMAPLLGRGKFEDLIKLPNDLDSVLPDYNFTVDNVGLAEANAHVWNAEAKGEVFTAEGYVLKPCYPLWLPNGNRVAIKCKNSKFSEKKKTDKPIKVAVVLSQDDLDLLQQFTDYVTVNRINNVISKIGEVSPKDFGKVMGLTVQDILEEAAREELELTDAENPVEVKKQLIECVKDTLRAVWIELVSK

SEQ ID NO: 10 - protein, 339 aa, Klebsiella phage KP27
MFKKYSSLTNHYEGKFINGVIMNGLTGGVWVAREKIHGANFSFITDDGITVTPAKRTDVVKPAEDFYGCSAVVAKYSPGIRKMWETLKKTGTYDDLVIQVYGEFAGRGVQKDVDYGEKDFYVFDIRVNGEFLPDNLCSLISRSHGLKMAPLLGYGTFEEIKELPITFESVVNKANSGIGSDNTVYGEFVYPIMDVEEGNIAEGFVMKPVSPAFMPNGERVAIKCKTTKFTEKKAKKATRFNAPVSLSEKDKNQLDEFVCYLTENRVKNVLSKLDLASITAKDFGRIMGLTVQDAIEEISRNHGPFLEQFEDPAMAKKLFVTEAQNMIRPVWGKILNHEF

SEQ ID NO: 11 - protein, 381 aa, Vibrio phage V05
MTTQELYNHLMTLTDDAEGKFFFADHISPLGEKLRVFSYHIASYSDWLLPGALEARGIMFQLDEQDKMVRIVSRPMEKFFNLNENPFTMDLDLTTTVQLMDKADGSLISTYLTGENFALKSKTSIFSEQAVAANRYIKLPENRDLWEFCDDLTQAGCTVNMEWCAPNNRIVLEYPEAKLVILNIRDNETGDYVSFDDIPLPALMRVKKWLVDEYDPETAHADDFVEKLRATKGIEGMILRLANGQSVKIKTQWYVDLHSQKDSVNVPKKLVTTILNNNHDDLYALFADDKPTIDRIREFDSHVSKTVSASFHAVSQFYVKNRHMSRKDYAIAGQKTLKPWEFGVAMIAYQNQTVEGVYEALVGAYLKRPELLIPEKYLNEA

SEQ ID NO: 12 - protein, 438 aa, Rhodothermus phage RM378
MESMNVKYPVEYLIEHLNSFESPEVAVESLRKEGIMCKNRGDLYMFKYHLGCKFDKIYHLACRGAILRKTDSGWKVLSYPFDKFFNWGEELQPEIVNYYQTLRYASPLNEKRKAGFMFKLPMKLVEKLDGTCVVLYYDEGWKIHTLGSIDANGSIVKNGMVTTHMDKTYRELFWETFEKKYPPYLLYHLNSSYCYIFEMVHPDARVVVPYEEPNIILIGVRSVDPEKGYFEVGPSEEAVRIFNESGGKINLKLPAVLSQEQNYTLFRANRLQELFEEVTPLFKSLRDGYEVVYEGFVAVQEIAPRVYYRTKIKHPVYLELHRIKTTITPEKLADLFLENKLDDFVLTPDEQETVMKLKEIYTDMRNQLESSFDTIYKEISEQVSPEENPGEFRKRFALRLMDYHDKSWFFARLDGDEEKMQKSEKKLLTERIEKGLFK

SEQ ID NO: 13 - protein, 376 aa, Citrobacter phage CkP1
MKKLFKNLMALCDEADESKFFYRDDISPSGLKYRIFSYNYASYSDWIRPDALECRGIMFEMIDDKPVRIASRPMEKFFNLNETPFTMNLDLSKAKYMLDKADGSLVSTFLDGNILKFKSKSSIKSEQSYFSTAMLTESRHEALLARLLDLASDGFTANFEYVSPDNRIVLPYQEKQLILLNIRDNDTGEYVDYEDIFKDGVLRQYLVQRHEITDSNFVEDIRKLTDIEGFVFVMEDGLRFKLKTDWYCALHHTKDSITNNERLFESIVNNASDDLKAMFAGDEFAVNKINKFEENYLKYLGESLHLINTTYHELRGRDRKDYAIESQNRANKSGLGFLFSIIMKMYNGGMDHDTRVKNLSELFMKNYKQFVPKEFI

SEQ ID NO: 14 - protein, 374 aa, Escherichia phage JN02
MEKLYYNLLSLCKSSSDRKFFYSDDVSPIGKKYRIFSYNFASYSDWLLPDALECRGIMFEMDGETPVRIASRPMEKFFNLNENPFTLSINLDDVKYLMTKEDGSLVSTYLDGGTVRFKSKGSIKSDQAVSATSILLDIDHKNLADRLLELCNDGFTANFEYVAPTNKIVLTYPEKRLILLNIRDNNTGEYIEYDDIYLDPVFRKYLVDRFEVPEGDWTSDVKSSTNIEGYVAVMKDGSHFKLKTDWYVALHTTRDSISSPEKLFLAIVNGASDDLKAMYADDEFSFKKVELFEKAYLDFLDRSFYICLDTYDKHKGKDRKTYAIEAQAVCKGAQTPWLFGIIMNLYQGGSKEQMMTALESVFIKNHKNFIPEGY

SEQ ID NO: 15 - protein, 383 aa, Klebsiella phage KP179
MLELYKNLMNLCESSEVAKFFYKDFTGPMDGKFRVFSYHYASYSEWLKPDALECRGIMFEMDGDTPIRIASRPMEKFFNLNENPLTMGIDISDVEYIMDKADGSLVSSYVDDGYLYLKSKTSLYSDQARQASALLNSEEYSSLHQVILELTLDGYTVNMEFVSPNNRVVLAYQEPQLFVLNVRNNTTGEYIKYDDLYANAKIRPYLINAYGISDPTTWVEGVRELEGVEGYIAVLNTGQRFKVKTEWYSALHHTKDSITSNERLFASVVSANSDDLRSLFAGDEYAIKKISAFEQAYLDYLGKSLELCQSFYDEYRGRARKDYAIAAQKATVNQRHLFGVIMNMYEGTVDVDKLLKDLERVFLKYWAGYVPKEYEKEIELSEE

SEQ ID NO: 16 - protein, 379 aa, Vibrio phage nt-1
MNELYNNLMTLAESAEGKFFFADHLSPQGEKFRVFSYHIASYSDWLLPDALEARGIMFQLDENDEMIRIVSRPMEKFFNLGENPFTMDLDLTTTVQLMDKADGSLISTYLTGDNFALKSKTSIYSEQAVAANRYIKHVDNRDLWEFCDDCAAQNFTVNMEWCAPNNRIVLEYTEPKLIILNIRDNETGQYVSFDDIPIGALTRIKKWLVDEYDPMTAHVDDFVETLKAKKGIEGMILRLASGQSVKIKTTWYVDLHAQKDSVNSPKKLVTTILNKNHDDLYALFADDKPTIERIREFDDHVSKKVVESFHAVSQYYTKNRHLSRKDFAIAGQKALKPWEFGVAMIAYQNQTVEGVVTMLINAYLKRPELLIPEKYLSEV

SEQ ID NO: 17 - protein, 335 aa, Vibrio phage VH7D
MSFVKYTSLENSYRQAFVDKCDMLGVKEWVALEKIHGANFSFIVEFKPSTEEVPGEMSVTPAKRTSTIGANAMGDYDFYGCTSVVEAHIEKMQDISNWLFANDFIKNDETIIVYGELAGKGIQKEVNYGDKDFWAYDILCPETGEFLDWDVVLKACKFAGVKTTHEIARGTLDELLKIDPLFRSFHTPADVDSENVAEGFVVKQLKAEKRLHNGSRAILKVKNEKFKEKKNKQGKTPRAKVVLTEEQEKLHAAFSCYLTENRLRNVLSKIGKVEAKQFGMVSGLFVKDAKDEFERDERDEVAIPRDDWDVIKRSLVNVANEILRKNWLNIVDGTF

SEQ ID NO: 18 - protein, 339 aa, Klebsiella phage KP15
MFKKYSSLTNHYEGKFINGVIMNGLTGGVWVAREKIHGANFSFITDDGITVTPAKRTDVVKPAEDFYGCSAVVAKYSPGIRKMWETLKKTGTYDDLVIQVYGEFAGRGVQKDVDYGEKDFYVFDIRVNGEFLPDNLCSLISRSHGLKMAPLLGYGTFEEIKELPITFESVVNKANSGIGSDNTVYGEFVYPIMDVEEGNIAEGFVMKPVSPAFMPNGERVAIKCKTTKFTEKKAKKATRFNAPVSLSEKDKNQLDEFVCYLTENRVKNVLSKLDLASITAKDFGRIMGLTVQDAIEEISRNHGPFIEQFEDPAMAKKLFVTEAQNMIRPVWGKILNHEF

SEQ ID NO: 19 - protein, 335 aa, Vibrio phage JN02
MFKKYSSLENHYNSKFIEKLYTNGLTTGVWVAREKIHGTNFSLIIERDNVTCAKRTGPILPAEDFYGYEIVLKKYDKAIKAVQEVMESISTSVPVSYQVFGEFAGGGIQKGVDYGEKDFYVFDIIINTESDDTYYMSDYEMQDFCNTFGFKMAPMLGRGTFDSLIMIPNDLDSVLAAYNSTASEDLVEANNCVFDANVIGDNTAEGYVLKPCFPKWLSNGTRVAIKCKNSKFSEKKKSDKPVKTQVPLTEIDKNLLDVLACYVTLNRVNNVISKIGTVTPKDFGKVMGLTVQDILEETSREGIVLTSSDNPNLVKKELVRMVQDVLRPAWIELVS

SEQ ID NO: 20 - protein, 334 aa, Escherichia phage JS98
MFKKYSSLENHYNSKFIEKLRTNGLTGGEWVAREKIHGTNFSLIIERDAVTCAKRTGPILPAEDFYGYEIVLKNYADSIKSVQHLIESINYQSYQIYGELAGPGIQKNVDYGDKDFYVFDIRVTKEDGTESVLTDTLMEAFCIIHKFKVAPCLATGSFEDLIKLPNDFDSVIPDYNFAVDNAGLTIANSTDFIPKVEGKVFTAEGFVLKPDIPTWLPNGNRVAIKCKNSKFSEKKKSDKPIKAAVVLSQDDMDLMWQFTDYVTVNRINNVISKIGEVSKKDFGKVMGLTVQDILEEAAREELELTDAENPVEVKKQLVECVKDTLRAVWIELVS

SEQ ID NO: 21 - protein, 379 aa, Escherichia phage JS98
MVSSVYKEILVKLGLTEDRIETLEMKGGIIEDEFDGIRYVRFKDSAGKLRRGTVVIDEEYVIPGFPHIKRIINLRSGIRRIFKRGEFYVEEKVDGYNVRVVMYKGKMLGITRGGFICPFTTERIPDFVPQEFFKDNPNLILVGEMAGPESPYLVEGPPYVKEDIQFFLFDVQEIKTGRSLPVEERLKIAEEYGINHVEVFGKYTKDDVDELYQLIERLSKEGREGIIMKSPDMKKIVKYVTPYANINDIKIGARVFYELPPGYFTSRISRLAFYLAEKRIKGEEFERVAKELGSALLQPFVESIFDVEQEEDIHELFKVRVKRIETAYKMVTHFEKLGLKIEIVDIEEIKDGWRITFKRLYPDATNEIRELIGGKAFVD

SEQ ID NO: 22 - protein, 342 aa, fungus Deinococcus radiodurans
MAERQVIKERAQLFPHPNAERLELCKVGTFQLVVRKGEYRDGDPIVIAPEKAVLPPQLAGLYTNADTGASYLHGAEKNRVGSVRLRGEVSQGVILPLDGLEDAPFGEDLAERLGITFWEPPVPVSMAGEVEPRPPAQHYKHHDVEQFGIYVSEFASGEEVMVTEKLHGTQGVYFRTAEGRWLVTSKGLSRGGLTLREAASNVYWQAARNSNLFAEADAAFSGGEVQIFGEVVPVQKGFSYGQHKPTVFVFKVVYDGLRLPRRDWPQWVLDHAVPVLYEGPFDEATVRKLRGGLETVSGKGLHIREGVVVAPKVPRFAADGSDLSVKLISDAYAKKETGEEYS

SEQ ID NO: 23 - RNA, 13 nt, synthetic construct
  source 1..13: mol_type = other RNA; note = F1
tccttagtcagta

SEQ ID NO: 24 - RNA, 10 nt, synthetic construct
  source 1..10: mol_type = other RNA; note = sF2
gatattttat

SEQ ID NO: 25 - RNA, 15 nt, synthetic construct
  source 1..15: mol_type = other RNA; note = P14
actcagtgaccccgt

SEQ ID NO: 26 - RNA, 15 nt, synthetic construct
  source 1..15: mol_type = other RNA; note = P13
acggggtcactgagt

SEQ ID NO: 27 - RNA, 10 nt, synthetic construct
  source 1..10: mol_type = other RNA; note = SN-2
ataatgctgg

SEQ ID NO: 28 - DNA, 16 bp, synthetic construct
  source 1..16: mol_type = other DNA; note = Nus-R
agcattatgaaagtga

SEQ ID NO: 29 - RNA, 12 nt, synthetic construct
  source 1..12: mol_type = other RNA; note = d1
tactctgagtct

SEQ ID NO: 30 - RNA, 14 nt, synthetic construct
  source 1..14: mol_type = other RNA; note = d4
aatatcaatagact

SEQ ID NO: 31 - RNA, 24 nt, synthetic construct
  source 1..24: mol_type = other RNA; note = C1
gactgacagatggcctataacgtg